European Patent Application EP 4 640 830 A1, published October 29, 2025. Title: MEANS AND METHODS FOR SAFE AND EFFICIENT GENE EDITING IN CELLS. Applicant: FONDAZIONE TELETHON ETS. The sequence listing filed with the application follows.

SEQUENCE LISTING (56 sequences)

SEQ ID NO: 1 - DNA, 20 bp, synthetic construct
  source 1..20: mol_type = other DNA
aaacgcaggccttacctgtc

SEQ ID NO: 2 - DNA, 20 bp, synthetic construct
  source 1..20: mol_type = other DNA
gtcagtttgcggccgctgtg

SEQ ID NO: 3 - DNA, 20 bp, synthetic construct
  source 1..20: mol_type = other DNA
tacccccagcttccacagcg

SEQ ID NO: 4 - DNA, 20 bp, synthetic construct
  source 1..20: mol_type = other DNA
ttgttggcagctgccacctg

SEQ ID NO: 5 - DNA, 20 bp, synthetic construct
  source 1..20: mol_type = other DNA
tagacgagggcctttactcc

SEQ ID NO: 6 - DNA, 20 bp, synthetic construct
  source 1..20: mol_type = other DNA
agtgaagcagacatagacga

SEQ ID NO: 7 - DNA, 20 bp, synthetic construct
  source 1..20: mol_type = other DNA
acgcgacgtttcttggacag

SEQ ID NO: 8 - DNA, 20 bp, synthetic construct
  source 1..20: mol_type = other DNA
tcagcatgtttcccgacatc

SEQ ID NO: 9 - DNA, 20 bp, synthetic construct
  source 1..20: mol_type = other DNA
caccttgtttactctactca

SEQ ID NO: 10 - DNA, 20 bp, synthetic construct
  source 1..20: mol_type = other DNA
aacaaagcagataatgatgc

SEQ ID NO: 11 - DNA, 20 bp, synthetic construct
  source 1..20: mol_type = other DNA
aatgctattgtgcaatccgt

SEQ ID NO: 12 - DNA, 20 bp, synthetic construct
  source 1..20: mol_type = other DNA
aatagcttcatagccaacat

SEQ ID NO: 13 - DNA, 20 bp, synthetic construct
  source 1..20: mol_type = other DNA
ctagaggaacatgccatcgc

SEQ ID NO: 14 - DNA, 20 bp, synthetic construct
  source 1..20: mol_type = other DNA
aagttgctaagttggacacg

SEQ ID NO: 15 - DNA, 20 bp, synthetic construct
  source 1..20: mol_type = other DNA
ggatttgaaccacatgcaag

SEQ ID NO: 16 - DNA, 20 bp, synthetic construct
  source 1..20: mol_type = other DNA
agggccttctggacaagcat

SEQ ID NO: 17 - DNA, 20 bp, synthetic construct
  source 1..20: mol_type = other DNA
gcccgttaccaatgcgcgag

SEQ ID NO: 18 - DNA, 20 bp, synthetic construct
  source 1..20: mol_type = other DNA
ctgccaggcatcgagcccac

SEQ ID NO: 19 - DNA, 20 bp, synthetic construct
  source 1..20: mol_type = other DNA
cgaggtgacggggactcata

SEQ ID NO: 20 - DNA, 20 bp, synthetic construct
  source 1..20: mol_type = other DNA
tcacaatcagaataacgagc

SEQ ID NO: 21 - DNA, 20 bp, synthetic construct
  source 1..20: mol_type = other DNA
gaataacgagcaggcttgga

SEQ ID NO: 22 - DNA, 20 bp, synthetic construct
  source 1..20: mol_type = other DNA
ggatgaggatatcagtcaga

SEQ ID NO: 23 - DNA, 20 bp, synthetic construct
  source 1..20: mol_type = other DNA
aaggccgtcagttcatcctg

SEQ ID NO: 24 - DNA, 20 bp, synthetic construct
  source 1..20: mol_type = other DNA
ctcagagattgctgcatagt

SEQ ID NO: 25 - DNA, 20 bp, synthetic construct
  source 1..20: mol_type = other DNA
cgtcagcttcaatcctgcca

SEQ ID NO: 26 - DNA, 20 bp, synthetic construct
  source 1..20: mol_type = other DNA
tccctgttctcgtttgatat

SEQ ID NO: 27 - DNA, 20 bp, synthetic construct
  source 1..20: mol_type = other DNA
ggatatagcatactatgatg

SEQ ID NO: 28 - DNA, 20 bp, synthetic construct
  source 1..20: mol_type = other DNA
gctcaaagccctgggtcgct

SEQ ID NO: 29 - DNA, 20 bp, synthetic construct
  source 1..20: mol_type = other DNA
ccagctcatcaataatatgc

SEQ ID NO: 30 - DNA, 20 bp, synthetic construct
  source 1..20: mol_type = other DNA
gctcataaggactaccgact

SEQ ID NO: 31 - DNA, 20 bp, synthetic construct
  source 1..20: mol_type = other DNA
gcacaccatcaggccggcct

SEQ ID NO: 32 - DNA, 20 bp, synthetic construct
  source 1..20: mol_type = other DNA
cgactctcggattatagcat

SEQ ID NO: 33 - DNA, 20 bp, synthetic construct
  source 1..20: mol_type = other DNA
gttcgatgtcgtccagcgtc

SEQ ID NO: 34 - DNA, 20 bp, synthetic construct
  source 1..20: mol_type = other DNA
agatagttaagtggggtaag

SEQ ID NO: 35 - DNA, 20 bp, synthetic construct
  source 1..20: mol_type = other DNA
gtcaccaatcctgtccctag

SEQ ID NO: 36 - DNA, 16 bp, synthetic construct
  source 1..16: mol_type = other DNA
tcccgacaattgtaag

SEQ ID NO: 37 - DNA, 408 bp, synthetic construct
  source 1..408: mol_type = other DNA
gtaacgccattttgcaaggcatggaaaaataccaaaccaagaatagagaagttcagatcaagggcgggtacatgaaaatagctaacgttgggccaaacaggatatctgcggtgagcagtttcggccccggcccggggccaagaacagatggtcaccgcagtttcggccccggcccgaggccaagaacagatggtccccagatatggcccaaccctcagcagtttcttaagacccatcagatgtttccaggctcccccaaggacctgaaatgaccctgcgccttatttgaattaaccaatcagcctgcttctcgcttctgttcgcgcgcttctgcttcccgagctctataaaagagctcacaacccctcactcggcgcgccagtcctccgacagactgagtcgcccggg

SEQ ID NO: 38 - DNA, 720 bp, synthetic construct
  source 1..720: mol_type = other DNA
atggtgagcaagggcgaggagctgttcaccggggtggtgcccatcctggtcgagctggacggcgacgtaaacggccacaagttcagcgtgtccggcgagggcgagggcgatgccacctacggcaagctgaccctgaagttcatctgcaccaccggcaagctgcccgtgccctggcccaccctcgtgaccaccctgacctacggcgtgcagtgcttcagccgctaccccgaccacatgaagcagcacgacttcttcaagtccgccatgcccgaaggctacgtccaggagcgcaccatcttcttcaaggacgacggcaactacaagacccgcgccgaggtgaagttcgagggcgacaccctggtgaaccgcatcgagctgaagggcatcgacttcaaggaggacggcaacatcctggggcacaagctggagtacaactacaacagccacaacgtctatatcatggccgacaagcagaagaacggcatcaaggtgaacttcaagatccgccacaacatcgaggacggcagcgtgcagctcgccgaccactaccagcagaacacccccatcggcgacggccccgtgctgctgcccgacaaccactacctgagcacccagtccgccctgagcaaagaccccaacgagaagcgcgatcacatggtcctgctggagttcgtgaccgccgccgggatcactctcggcatggacgagctgtacaagtaa

SEQ ID NO: 39 - DNA, 225 bp, synthetic construct
  source 1..225: mol_type = other DNA
ctgtgccttctagttgccagccatctgttgtttgcccctcccccgtgccttccttgaccctggaaggtgccactcccactgccctttcctaataaaatgaggaaattgcatcgcattgtctgagtaggtgtcattctattctggggggtggggtggggcaggacagcaagggggaggattgggaagacaatagcaggcatgctggggatgcggtgggctctatgg

SEQ ID NO: 40 - DNA, 500 bp, synthetic construct
  source 1..500: mol_type = other DNA
gtgcaaatcagaccacctgggttcagatcttaggtctgacagctgtgttaccctgggcaagtcctcacctttctgtgcctgtcccctctttgctgtaaaatgggggtactaatacttaagtcttcccttcccccacagttgctactaacaaacagaaaaacggtacccatgtgctccagggtcacctctgacctttttttcctccagatgtccagctcgccgctgtccaagaaacgtcgcgtgtccgggcctgatccaaagccgggttctaactgctcccctgcccagtccgtgttgtccgaagtgccctcggtgccaaccaacgtgagtgtcctctccgtggagactggcagacgaggtggtgggtgggaaagtcttttgtatcactgtctgtctatccatgctccactcctgtgtgtctccctaaacttgttcttttcctctattcctagggaatggccaagaacggcagtgaagcagacatagacgagggcctttac

SEQ ID NO: 41 - DNA, 800 bp, synthetic construct
  source 1..800: mol_type = other DNA
tggggccaaggccgggctgaggggtgtggaatgggacattgagaggataaggttgggtggggcaggccctgacctagagtaccccctaacctggcaggtatgtgttgggccatgaggcaatgaagcggctccagacatccagtgtcctggtatcaggcctgcggggcctgggcgtggagatcgctaagaacatcatccttggtggggtcaaggctgttaccctacatgaccagggcactgcccagtgggctgatctttcctcccaggtacctcttcctagcacccttccccctttcccccttcccgaggcaccactgttcccggtgccacagccatttcatctttttccctactgcacacccttacagttctacctgcgggaggaggacatcggtaaaaaccgggccgaggtatcacagccccgcctcgctgagctcaacagctatgtgcctgtcactgcctacactggacccctcgttgaggacttccttagtggtttccaggtatcttgggggtactacccagccttctgcccagttttctcagagcccatctctggtttattcagtagtgttcaatattgatttaatgggtcggcctgaatgtcaggttttgtgctgggggactagagtatgcaggcagcagttagcccctggccctgccttttcttttcttctttttttttttttgagacggagtcttgctctgtcgcccaagctagagtgcagtggcgcgatctcggctcactgcaagctacacctcctgggttcacgccattctcctgcctcagcctcccgagt

SEQ ID NO: 42 - DNA, 26 bp, synthetic construct
  source 1..26: mol_type = other DNA
aggtggccgccgctaacaagaagcac

SEQ ID NO: 43 - DNA, 26 bp, synthetic construct
  source 1..26: mol_type = other DNA
aggtggccgccgctaacaagaagcac

SEQ ID NO: 44 - DNA, 500 bp, synthetic construct
  source 1..500: mol_type = other DNA
cttgaggcccggtcatcaattccccaacgaatggtcctgcatagtctgcccagcccctcaggcccctcctatcagaggcaggcaggaggggattctgcagaaaagcaaacagcacggggcctcaccccgacctctctggctgactagcccaggctccaggagggtaatttagcgactatctgctttcattagcctgctcgttaacttttcccaattgatttttcggggcttttgatctaaatgcttgcacaaacaacaccccgtcagctcccaggggggctcccactactgcccccagctcgttagaatgcacctgactagggccctcagtgggacttggctggcggcaggtggctttttgagaagcctggctcacagccaggagggaaggggctgagaacaggacctgtgctcactggggcctgcatgacccttccctccccacagcggccgcaaactgacacctcagggacaaagagatctggacagaatcgccggac

SEQ ID NO: 45 - DNA, 500 bp, synthetic construct
  source 1..500: mol_type = other DNA
aggtaaggcctgcgtttggggtggggctgggtcccttagtcgctgcccaagcatttccaaagcccatactttgtcaggtagacttatttccttctctggagggcacagcccagggtgctggtggggtcagaggagggctgcccagagacaggagaaaggacagtcctgtctgacttttcctgttggtgctgcttagaaatttggaggcaggctggctgtggtgtctcacccctgtaatcccagcactttgggatgccgaggcaggcgaattatctgaggtcaggagttcaagaccattctgaccaacatggagaaaccctgtctctactaaaaatacaaaattagccgggtgtggtggcacattcctgtaatctcagctactggggaggctgaggcacaaaaatcacttgaacccgggaggtggaggctgcggtgagccaagatcatgccattgcaccccagcctgggcaacaagagtgaaactccatctcaaaaaaaaa

SEQ ID NO: 46 - DNA, 26 bp, synthetic construct
  source 1..26: mol_type = other DNA
aggtggccgccgctaacaagaagcac

SEQ ID NO: 47 - DNA, 500 bp, synthetic construct; identical to SEQ ID NO: 44
  source 1..500: mol_type = other DNA

SEQ ID NO: 48 - DNA, 500 bp, synthetic construct; identical to SEQ ID NO: 45
  source 1..500: mol_type = other DNA

SEQ ID NO: 49 - DNA, 86 bp, synthetic construct
  source 1..86: mol_type = other DNA
cactcaatgttgtacccattgagccacggatttcgcaaagcaatagcagaacgtcatgggaatttatgtctagacaaggtgtgatt

SEQ ID NO: 50 - DNA, 500 bp, synthetic construct
  source 1..500: mol_type = other DNA
cttccattcataaggtactactgtttattataatatgtgcagtttaacacctaaaatttaacttttggaaattttttaccatcctgctttatttattttccaggattcagggaatattccagaagccatagcttcttaccgcacggctctgaaacttaagcctgattttcctgatgcttattgtaacttggctcattgcctgcaggtaaagaataacaggccagtaattggctctcagtgttgtaatagctttttaattgttgtatgccataagaatccaagcctgactggaaatagtatttttaataggctatctgacattactttaggccaaagacatatcaaatattaaatcctgggataggactttctggataataacttgtttttgctttctctagattgtctgtgattggacagactatgatgagcgaatgaagaagttggtcagtattgtggctgaccagttagagaagaataggttgccttctgtgcatcct

SEQ ID NO: 51 - DNA, 900 bp, synthetic construct
  source 1..900: mol_type = other DNA
cttttgttttaatctttttgttgtaaactaaaacacaaatacagaaaactgtaaaaatcaaatctgtggcttaatgaacgattataaagtgaacaccacccaagtcgagaaataaaacttttgtgggccacttcagaaccccttccattgtgtcctgagtataaccccctgcacttcataagacggaatccttaactccttcacttaaacactaatgatagactgatggtacttttctttaagttgaaagccataatttttttttcttttatcttttttttcttttttttttgagacggggtcttgctctgtcgcccaggctggagtgcagcggtgtgatcatggcttactgcagccttgacctccccgagcttaggtgatcctcccacctcagcctcctgagtagctgggactacaggcgcatgccaccacacctaattttgtgttttttgtagagatggggttttgctatgttgcccaagctggtcttgaacctctgggctcaagtgatctgcccacctcgcccggccaaagtgctgggattacgggtgtgagccaccgcgcctggccagccatcatgtttaatggagtgcttggtattttgtattcacctttgagaattagagcagtacttgatcaaggattggatcaaaggttggataatagattggagtgctaggtgtactttttttttttttttgagacatagtgtctctgtcatccagactgcagtgcagtggtgccatctcagctcattgcaacctctgtctcccaggttaaagtgatgctcgtgccttagcttcccgaggagctaggattacaggcgtgtgccaccacgcctggctaatttttgtatttttagtagagatagggctttgccatgctaggctggtctcgaaa

SEQ ID NO: 52 - DNA, 225 bp, synthetic construct
  source 1..225: mol_type = other DNA
ccatagagcccaccgcatccccagcatgcctgctattgtcttcccaatcctcccccttgctgtcctgccccaccccaccccccagaatagaatgacacctactcagacaatgcgatgcaatttcctcattttattaggaaagggcagtgggagtggcaccttccagggtcaaggaaggcacgggggaggggcaaacaacagatggctggcaactagaaggcacag

SEQ ID NO: 53 - DNA, 720 bp, synthetic construct
  source 1..720: mol_type = other DNA
ttacttgtacagctcgtccatgccgagagtgatcccggcggcggtcacgaactccagcaggaccatgtgatcgcgcttctcgttggggtctttgctcagggcggactgggtgctcaggtagtggttgtcgggcagcagcacggggccgtcgccgatgggggtgttctgctggtagtggtcggcgagctgcacgctgccgtcctcgatgttgtggcggatcttgaagttcaccttgatgccgttcttctgcttgtcggccatgatatagacgttgtggctgttgtagttgtactccagcttgtgccccaggatgttgccgtcctccttgaagtcgatgcccttcagctcgatgcggttcaccagggtgtcgccctcgaacttcacctcggcgcgggtcttgtagttgccgtcgtccttgaagaagatggtgcgctcctggacgtagccttcgggcatggcggacttgaagaagtcgtgctgcttcatgtggtcggggtagcggctgaagcactgcacgccgtaggtcagggtggtcacgagggtgggccagggcacgggcagcttgccggtggtgcagatgaacttcagggtcagcttgccgtaggtggcatcgccctcgccctcgccggacacgctgaacttgtggccgtttacgtcgccgtccagctcgaccaggatgggcaccaccccggtgaacagctcctcgcccttgctcaccat

SEQ ID NO: 54 - DNA, 408 bp, synthetic construct
  source 1..408: mol_type = other DNA
cccgggcgactcagtctgtcggaggactggcgcgccgagtgaggggttgtgagctcttttatagagctcgggaagcagaagcgcgcgaacagaagcgagaagcaggctgattggttaattcaaataaggcgcagggtcatttcaggtccttgggggagcctggaaacatctgatgggtcttaagaaactgctgagggttgggccatatctggggaccatctgttcttggcctcgggccggggccgaaactgcggtgaccatctgttcttggccccgggccggggccgaaactgctcaccgcagatatcctgtttggcccaacgttagctattttcatgtacccgcccttgatctgaacttctctattcttggtttggtatttttccatgccttgcaaaatggcgttac

SEQ ID NO: 55 - DNA, 407 bp, synthetic construct
  source 1..407: mol_type = other DNA
ctgcatttatttagtctccagaaaaaggggggaatgaaagaccccacctgtaggtttggcaagctaggatcaaggttaggaacagagagacagcagaatatgggccaaacaggatatctgtggtaagcagttcctgccccggctcagggccaagaacagttggaacagcagaatatgggccaaacaggatatctgtggtaagcagttcctgccccggctcagggccaagaacagatggtccccagatgcggtcccgccctcagcagtttctagagaaccatcagatgtttccagggtgccccaaggacctgaaatgaccctgtgccttatttgaactaaccaatcagttcgcttctcgcttctgttcgcgcgcttctgctccccgagctcaataaaagagcccaggg

SEQ ID NO: 56 - DNA, 1812 bp, synthetic construct
  source 1..1812: mol_type = other DNA
cagaaaaggagaagtaggagccaagatttccaaactctgtggttgccttgccaagatttccaaactctgtggttgccttgcagaaaaggagaagtaggagaagcgacttcctctttccagaagcgacttcctctttccagaggaagagggcggaggctcacaaggcaaccacagagtttggaaatcttggaagcgacttcctctttccagcagaaaaggagaagtaggagaagcgacttcctctttccaggtccgccctcgctagatctttattctgtttttaaattttttatttttatattttacctttaaaacatttttgttaaaagctaagacacaaacatacacattagcctaggcccacacaaagtcaggatcattaatatcactgtcttccacctccacattttgccccactggacagtcttcaagggcactaacatgcatgaagctgtcatctatgacagcaatgcattcttctggaataccttctgaaggacctgcctgagattcttttacagttaacttttttataagtaggagtatactctaaaataatgattaaaagtatagtctagtaaataaatgaaccagtaacatagtcatctatttttactatcaagtactatgtaatgtacataattgtatgtgctatacttttacaactggcagctcagtaggtttgtttacaccagcattgccacaaacacatgagtaatgtgttatgctacaatgtcactagatggtaggaatttttcagcacacacacacaagtatatatattatatattatattatatattatatatatatatgtatatatatatatatatatagagagagagagagagagagagagagagagatggagtcttgctctgtcgcccaggctggggtgcaatgacacaatctcggctcactgcaacctgactcccaggttcaagtgattctcctgcctcagcctcctgagtagctgggactacaggtgcccaccaccatgcccagctaatttttgtatttttagtagagacggggtttcaccatgttggccagattggtcccaaactcctgacctcaagtgatccaccccactcagcctctcaaagtgctgggattacaggcgtgagccaccgtgcctggccaacaccattataatcttatgggaccactgtcatacatgtggttcatcattggccaaagcatctgtatttatatatgtatgtttcaaattatatatatatatatatatatatatatatatgatagctatacatgaacatacacacacacatatatagacatatatagcacataaaattggcacatattaagcattttgtaaatatcaaccattacaattgttactacttttctcagcaaggctatgaatgctgttccagcctgtcaaaatcacacctgtttaatgtgttttacccagcacgaagtcatgtctagttgagtggcttaaaaattgtgatcaaatagctggttagttaaaaagttatttcactgtgtaaaatacatcccttaaaatgcactgttatttatctcttagttgtagaaattggtttcattttccactatgtttaattgtgactggatcattatagaccctttttttgtagttgttgaggtttaaagatttaagtttgttatggatgcaagcttttcagttgaccaatgattattagccaatttctgataaaagaaaaggaaaccgattgccccagggctgctgttttcatttcctcattggaagaagaagcatagtatagaagaaaggcaaacacaacacattcaacctctgccacc